European Patent Specification EP 3 353 204 B1, published October 18, 2023. Title: METHODS AND COMPOSITIONS FOR TREATMENT OF CANCER. Applicant: OncoMed Pharmaceuticals, Inc. Dupont, Jakob Parmar, Hema Stagg, Robert J. The sequence listing filed with the application follows.

SEQUENCE LISTING (80 sequences)

SEQ ID NO: 1 - protein, 464 aa, Artificial Sequence
  21M18 Heavy chain
  SIGNAL (1)..(19)
MKHLWFFLLLVAAPRWVLSQVQLVQSGAEVKKPGASVKISCKASGYSFTAYYIHWVKQAPGQGLEWIGYISSYNGATNYNQKFKGRVTFTTDTSTSTAYMELRSLRSDDTAVYYCARDYDYDVGMDYWGQGTLVTVSSASTKGPSVFPLAPCSRSTSESTAALGCLVKDYFPEPVTVSWNSGALTSGVHTFPAVLQSSGLYSLSSVVTVPSSNFGTQTYTCNVDHKPSNTKVDKTVERKCCVECPPCPAPPVAGPSVFLFPPKPKDTLMISRTPEVTCVVVDVSHEDPEVQFNWYVDGVEVHNAKTKPREEQFNSTFRVVSVLTVVHQDWLNGKEYKCKVSNKGLPAPIEKTISKTKGQPREPQVYTLPPSREEMTKNQVSLTCLVEGFYPSDIAVEWESNGQPENNYKTTPPMLDSDGSFFLYSELTVDKSRWQQGNVFSCSVMHEALHNHYTQKSLSLSPGK

SEQ ID NO: 2 - protein, 464 aa, Artificial Sequence
  21R79 Heavy chain
  SIGNAL (1)..(19)
MKHLWFFLLLVAAPRWVLSQVQLVQSGAEVKKPGASVKISCKASGYSFTAYYIHWVKQAPGQGLEWIGYIANYNRATNYNQKFKGRVTFTTDTSTSTAYMELRSLRSDDTAVYYCARDYDYDVGMDYWGQGTLVTVSSASTKGPSVFPLAPCSRSTSESTAALGCLVKDYFPEPVTVSWNSGALTSGVHTFPAVLQSSGLYSLSSVVTVPSSNFGTQTYTCNVDHKPSNTKVDKTVERKCCVECPPCPAPPVAGPSVFLFPPKPKDTLMISRTPEVTCVVVDVSHEDPEVQFNWYVDGVEVHNAKTKPREEQFNSTFRVVSVLTVVHQDWLNGKEYKCKVSNKGLPAPIEKTISKTKGQPREPQVYTLPPSREEMTKNQVSLTCLVEGFYPSDIAVEWESNGQPENNYKTTPPMLDSDGSFFLYSELTVDKSRWQQGNVFSCSVMHEALHNHYTQKSLSLSPGK

SEQ ID NO: 3 - protein, 466 aa, Artificial Sequence
  219R45 Heavy chain
  SIGNAL (1)..(19)
MKHLWFFLLLVAAPRWVLSQVQLVQSGAEVKKPGASVKVSCKASGYTFTNYWMHWVRQAPGQGLEWMGDINPSNGRTSYKEKFKRRVTLSVDKSSSTAYMELSSLRSEDTAVYFCTIHYDDKYYPLMDYWGQGTLVTVSSASTKGPSVFPLAPCSRSTSESTAALGCLVKDYFPEPVTVSWNSGALTSGVHTFPAVLQSSGLYSLSSVVTVPSSNFGTQTYTCNVDHKPSNTKVDKTVERKCCVECPPCPAPPVAGPSVFLFPPKPKDTLMISRTPEVTCVVVDVSHEDPEVQFNWYVDGVEVHNAKTKPREEQFNSTFRVVSVLTVVHQDWLNGKEYKCKVSNKGLPAPIEKTISKTKGQPREPQVYTLPPSREKMTKNQVSLTCLVKGFYPSDIAVEWESNGQPENNYKTTPPMLKSDGSFFLYSKLTVDKSRWQQGNVFSCSVMHEALHNHYTQKSLSLSPGK

SEQ ID NO: 4 - protein, 238 aa, Artificial Sequence
  Light chain
  SIGNAL (1)..(20)
MVLQTQVFISLLLWISGAYGDIVMTQSPDSLAVSLGERATISCRASESVDNYGISFMKWFQQKPGQPPKLLIYAASNQGSGVPDRFSGSGSGTDFTLTISSLQAEDVAVYYCQQSKEVPWTFGGGTKVEIKRTVAAPSVFIFPPSDEQLKSGTASVVCLLNNFYPREAKVQWKVDNALQSGNSQESVTEQDSKDSTYSLSSTLTLSKADYEKHKVYACEVTHQGLSSPVTKSFNRGEC

SEQ ID NO: 5 - protein, 445 aa, Artificial Sequence
  21M18 Heavy chain
QVQLVQSGAEVKKPGASVKISCKASGYSFTAYYIHWVKQAPGQGLEWIGYISSYNGATNYNQKFKGRVTFTTDTSTSTAYMELRSLRSDDTAVYYCARDYDYDVGMDYWGQGTLVTVSSASTKGPSVFPLAPCSRSTSESTAALGCLVKDYFPEPVTVSWNSGALTSGVHTFPAVLQSSGLYSLSSVVTVPSSNFGTQTYTCNVDHKPSNTKVDKTVERKCCVECPPCPAPPVAGPSVFLFPPKPKDTLMISRTPEVTCVVVDVSHEDPEVQFNWYVDGVEVHNAKTKPREEQFNSTFRVVSVLTVVHQDWLNGKEYKCKVSNKGLPAPIEKTISKTKGQPREPQVYTLPPSREEMTKNQVSLTCLVEGFYPSDIAVEWESNGQPENNYKTTPPMLDSDGSFFLYSELTVDKSRWQQGNVFSCSVMHEALHNHYTQKSLSLSPGK

SEQ ID NO: 6 - protein, 445 aa, Artificial Sequence
  21R79 Heavy chain
QVQLVQSGAEVKKPGASVKISCKASGYSFTAYYIHWVKQAPGQGLEWIGYIANYNRATNYNQKFKGRVTFTTDTSTSTAYMELRSLRSDDTAVYYCARDYDYDVGMDYWGQGTLVTVSSASTKGPSVFPLAPCSRSTSESTAALGCLVKDYFPEPVTVSWNSGALTSGVHTFPAVLQSSGLYSLSSVVTVPSSNFGTQTYTCNVDHKPSNTKVDKTVERKCCVECPPCPAPPVAGPSVFLFPPKPKDTLMISRTPEVTCVVVDVSHEDPEVQFNWYVDGVEVHNAKTKPREEQFNSTFRVVSVLTVVHQDWLNGKEYKCKVSNKGLPAPIEKTISKTKGQPREPQVYTLPPSREEMTKNQVSLTCLVEGFYPSDIAVEWESNGQPENNYKTTPPMLDSDGSFFLYSELTVDKSRWQQGNVFSCSVMHEALHNHYTQKSLSLSPGK

SEQ ID NO: 7 - protein, 447 aa, Artificial Sequence
  219R45 Heavy chain
QVQLVQSGAEVKKPGASVKVSCKASGYTFTNYWMHWVRQAPGQGLEWMGDINPSNGRTSYKEKFKRRVTLSVDKSSSTAYMELSSLRSEDTAVYFCTIHYDDKYYPLMDYWGQGTLVTVSSASTKGPSVFPLAPCSRSTSESTAALGCLVKDYFPEPVTVSWNSGALTSGVHTFPAVLQSSGLYSLSSVVTVPSSNFGTQTYTCNVDHKPSNTKVDKTVERKCCVECPPCPAPPVAGPSVFLFPPKPKDTLMISRTPEVTCVVVDVSHEDPEVQFNWYVDGVEVHNAKTKPREEQFNSTFRVVSVLTVVHQDWLNGKEYKCKVSNKGLPAPIEKTISKTKGQPREPQVYTLPPSREKMTKNQVSLTCLVKGFYPSDIAVEWESNGQPENNYKTTPPMLKSDGSFFLYSKLTVDKSRWQQGNVFSCSVMHEALHNHYTQKSLSLSPGK

SEQ ID NO: 8 - protein, 217 aa, Artificial Sequence
  Light chain
DIVMTQSPDSLAVSLGERATISCRASESVDNYGISFMKWFQQKPGQPPKLLIYAASNQGSGVPDRFSGSGSGTDFTLTISSLQAEDVAVYYCQQSKEVPWTFGGGTKVEIKRTVAAPSVIFPPSDEQLKSGTASVVCLLNNFYPREAKVQWKVDNALQSGNSQESVTEQDSKDSTYSLSSTLTLSKADYEKHKVYACEVTHQGLSSPVTKSFNRGEC

SEQ ID NO: 9 - protein, 119 aa, Artificial Sequence
  21M18 Heavy chain
QVQLVQSGAEVKKPGASVKISCKASGYSFTAYYIHWVKQAPGQGLEWIGYISSYNGATNYNQKFKGRVTFTTDTSTSTAYMELRSLRSDDTAVYYCARDYDYDVGMDYWGQGTLVTVSS

SEQ ID NO: 10 - protein, 119 aa, Artificial Sequence
  21R79 Heavy chain variable region
QVQLVQSGAEVKKPGASVKISCKASGYSFTAYYIHWVKQAPGQGLEWIGYIANYNRATNYNQKFKGRVTFTTDTSTSTAYMELRSLRSDDTAVYYCARDYDYDVGMDYWGQGTLVTVSS

SEQ ID NO: 11 - protein, 121 aa, Artificial Sequence
  219R45 Heavy chain variable region
QVQLVQSGAEVKKPGASVKVSCKASGYTFTNYWMHWVRQAPGQGLEWMGDINPSNGRTSYKEKFKRRVTLSVDKSSSTAYMELSSLRSEDTAVYFCTIHYDDKYYPLMDYWGQGTLVTVSS

SEQ ID NO: 12 - protein, 111 aa, Artificial Sequence
  Light chain variable region
DIVMTQSPDSLAVSLGERATISCRASESVDNYGISFMKWFQQKPGQPPKLLIYAASNQGSGVPDRFSGSGSGTDFTLTISSLQAEDVAVYYCQQSKEVPWTFGGGTKVEIK

SEQ ID NO: 13 - protein, 6 aa, Artificial Sequence
  21R75, 21R79, 21R83, and 21M18 Heavy chain CDR1
TAYYIH

SEQ ID NO: 14 - protein, 17 aa, Artificial Sequence
  21R79 Heavy chain CDR2
YIANYNRATNYNQKFKG

SEQ ID NO: 15 - protein, 17 aa, Artificial Sequence
  21M18 Heavy chain CDR2
YISSYNGATNYNQKFKG

SEQ ID NO: 16 - protein, 11 aa, Artificial Sequence
  21R75, 21R79, 21R83, and 21M18 Heavy chain CDR3
RDYDYDVGMDY

SEQ ID NO: 17 - protein, 5 aa, Artificial Sequence
  219R45 Heavy chain CDR1
NYWMH

SEQ ID NO: 18 - protein, 17 aa, Artificial Sequence
  219R45 Heavy chain CDR2
DINPSNGRTSYKEKFKR

SEQ ID NO: 19 - protein, 12 aa, Artificial Sequence
  219R45 Heavy chain CDR3
HYDDKYYPLMDY

SEQ ID NO: 20 - protein, 15 aa, Artificial Sequence
  Light chain CDR1
RASESVDNYGISFMK

SEQ ID NO: 21 - protein, 7 aa, Artificial Sequence
  Light chain CDR2
AASNQGS

SEQ ID NO: 22 - protein, 12 aa, Artificial Sequence
  Light chain CDR3
QQSKEVPWTFGG

SEQ ID NO: 23 - protein, 522 aa, Homo sapiens
  SIGNAL (1)..(26)
MAAASRSASGWALLLLVALWQQRAAGSGVFQLQLQEFINERGVLASGRPCEPGCRTFFRVCLKHFQAVVSPGPCTFGTVSTPVLGTNSFAVRDDSSGGGRNPLQLPFNFTWPGTFSLIIEAWHAPGDDLRPEALPPDALISKIAIQGSLAVGQNWLLDEQTSTLTRLRYSYRVICSDNYYGDNCSRLCKKRNDHFGHYVCQPDGNLSCLPGWTGEYCQQPICLSGCHEQNGYCSKPAECLCRPGWQGRLCNECIPHNGCRHGTCSTPWQCTCDEGWGGLFCDQDLNYCTHHSPCKNGATCSNSGQRSYTCTCRPGYTGVDCELELSECDSNPCRNGGSCKDQEDGYHCLCPPGYYGLHCEHSTLSCADSPCFNGGSCRERNQGANYACECPPNFTGSNCEKKVDRCTSNPCANGGQCLNRGPSRMCRCRPGFTGTYCELHVSDCARNPCAHGGTCHDLENGLMCTCPAGFSGRRCEVRTSIDACASSPCFNRATCYTDLSTDTFVCNCPYGFVGSRCEFPVG

SEQ ID NO: 24 - protein, 496 aa, Homo sapiens
SGVFQLQLQEFINERGVLASGRPCEPGCRTFFRVCLKHFQAVVSPGPCTFGTVSTPVLGTNSFAVRDDSSGGGRNPLQLPFNFTWPGTFSLIIEAWHAPGDDLRPEALPPDALISKIAIQGSLAVGQNWLLDEQTSTLTRLRYSYRVICSDNYYGDNCSRLCKKRNDHFGHYVCQPDGNLSCLPGWTGEYCQQPICLSGCHEQNGYCSKPAECLCRPGWQGRLCNECIPHNGCRHGTCSTPWQCTCDEGWGGLFCDQDLNYCTHHSPCKNGATCSNSGQRSYTCTCRPGYTGVDCELELSECDSNPCRNGGSCKDQEDGYHCLCPPGYYGLHCEHSTLSCADSPCFNGGSCRERNQGANYACECPPNFTGSNCEKKVDRCTSNPCANGGQCLNRGPSRMCRCRPGFTGTYCELHVSDCARNPCAHGGTCHDLENGLMCTCPAGFSGRRCEVRTSIDACASSPCFNRATCYTDLSTDTFVCNCPYGFVGSRCEFPVG

SEQ ID NO: 25 - protein, 128 aa, Homo sapiens
SGVFQLQLQEFINERGVLASGRPCEPGCRTFFRVCLKHFQAVVSPGPCTFGTVSTPVLGTNSFAVRDDSSGGGRNPLQLPFNFTWPGTFSLIIEAWHAPGDDLRPEALPPDALISKIAIQGSLAVGQN

SEQ ID NO: 26 - protein, 63 aa, Homo sapiens
WLLDEQTSTLTRLRYSYRVICSDNYYGDNCSRLCKKRNDHFGHYVCQPDGNLSCLPGWTGEYC

SEQ ID NO: 27 - protein, 232 aa, Homo sapiens
  SIGNAL (1)..(26)
MNFLLSWVHWSLALLLYLHHAKWSQAAPMAEGGGQNHHEVVKFMDVYQRSYCHPIETLVDIFQEYPDEIEYIFKPSCVPLMRCGGCCNDEGLECVPTEESNITMQIMRIKPHQGQHIGEMSFLQHNKCECRPKKDRARQEKKSVRGKGKGQKRKRKKSRYKSWSVYVGARCCLMPWSLPGPHPCGPCSERRKHLFVQDPQTCKCSCKNTDSRCKARQLELNERTCRCDKPRR

SEQ ID NO: 28 - protein, 206 aa, Homo sapiens
APMAEGGGQNHHEVVKFMDVYQRSYCHPIETLVDIFQEYPDEIEYIFKPSCVPLMRCGGCCNDEGLECVPTEESNITMQIMRIKPHQGQHIGEMSFLQHNKCECRPKKDRARQEKKSVRGKGKGQKRKRKKSRYKSWSVYVGARCCLMPWSLPGPHPCGPCSERRKHLFVQDPQTCKCSCKNTDSRCKARQLELNERTCRCDKPRR

SEQ ID NO: 29 - DNA, 1395 bp, Artificial Sequence
  21M18 Heavy chain
atgaagcacctgtggttctttctgctgctggtggccgctcccagatgggtgctgtcccaggtgcagctggtgcagtctggcgccgaagtgaagaaacctggcgcctccgtgaagatctcctgcaaggcctccggctactccttcaccgcttactacatccactgggtcaagcaggcccctgggcagggcctggaatggatcggctacatctcctcctacaacggcgccaccaactacaaccagaaattcaagggccgcgtgaccttcaccaccgacacctccacctccaccgcctacatggaactgcggtccctgcggagcgacgacaccgccgtgtactactgcgccagagactacgactacgacgtgggcatggactactggggccagggcaccctggtcaccgtgtcctctgcctccaccaagggcccatccgtgttccctctggccccttgctcccggtccacctctgagtctaccgccgctctgggctgcctggtgaaggactacttccctgagcctgtgaccgtgtcctggaactctggcgccctgacctctggcgtgcacaccttccctgccgtgctgcagtcctccggcctgtactccctgtctagcgtggtgaccgtgccttcctccaacttcggcacccagacctacacctgtaacgtggaccacaagccttccaacaccaaggtggacaagaccgtggagcggaagtgctgcgtggagtgccctccttgtcctgctcctcctgtggctggcccttctgtgttcctgttccctccaaagcctaaggacaccctgatgatctcccggacccctgaagtgacctgcgtggtggtggacgtgtcccacgaggaccctgaggtgcagttcaattggtacgtggacggcgtggaggtgcacaacgccaagaccaagcctcgggaggaacagttcaactccaccttccgggtggtgtctgtgctgaccgtggtgcaccaggactggctgaacggcaaagaatacaagtgcaaggtgtccaacaagggcctgcctgcccctatcgaaaagaccatcagcaagaccaagggccagcctcgcgagcctcaggtgtacaccctgcctcccagccgggaagaaatgaccaagaaccaggtgtccctgacctgtctggtggagggcttctacccttccgatatcgccgtggagtgggagtctaacggccagcctgagaacaactacaagaccacccctcctatgctggactccgacggctccttcttcctgtactccgaactgaccgtggacaagtcccggtggcagcagggcaacgtgttctcctgctccgtgatgcacgaggccctgcacaaccactacacccagaagtccctgtccctgtctcctggcaagtag

SEQ ID NO: 30 - DNA, 1395 bp, Artificial Sequence
  21R79 Heavy chain
atgaagcacctgtggttctttctgctgctggtggccgctcccagatgggtgctgtcccaggtgcagctggtgcagtctggcgccgaagtgaagaaacctggcgcctccgtgaagatctcctgcaaggcctccggctactccttcaccgcctactacatccactgggtgaaacaggcaccaggccagggactggaatggatcggctatatcgccaactacaaccgggccaccaactacaaccagaaattcaagggccgcgtgaccttcaccaccgacacctccacctccacagcctacatggaactgcggtccctgcggagcgacgacaccgccgtgtactactgcgccagagactacgactacgacgtgggcatggactactggggccagggcaccctggtgacagtgtcctccgcctccaccaagggcccctccgtgttccctctggccccttgctcccggtccacctctgagtctaccgccgctctgggctgcctggtgaaggactacttccctgagcctgtgaccgtgtcctggaactctggcgccctgacctctggcgtgcacaccttccctgccgtgctgcagtcctccggcctgtactccctgtctagcgtggtgaccgtgccttcctccaacttcggcacccagacctacacctgtaacgtggaccacaagccttccaacaccaaggtggacaagaccgtggagcggaagtgctgcgtggagtgccctccttgtcctgctcctcctgtggctggcccttctgtgttcctgttccctccaaagcctaaggacaccctgatgatctcccggacccctgaagtgacctgcgtggtggtggacgtgtcccacgaggaccctgaggtgcagttcaattggtacgtggacggcgtggaggtgcacaacgccaagaccaagcctcgggaggaacagttcaactccaccttccgggtggtgtctgtgctgaccgtggtgcaccaggactggctgaacggcaaagaatacaagtgcaaggtgtccaacaagggcctgcctgcccctatcgaaaagaccatcagcaagaccaagggccagcctcgcgagcctcaggtgtacaccctgcctcccagccgggaagaaatgaccaagaaccaggtgtccctgacctgtctggtggagggcttctacccttccgatatcgccgtggagtgggagtctaacggccagcctgagaacaactacaagaccacccctcctatgctggactccgacggctccttcttcctgtactccgaactgaccgtggacaagtcccggtggcagcagggcaacgtgttctcctgctccgtgatgcacgaggccctgcacaaccactacacccagaagtccctgtccctgtctcctggcaagtag

SEQ ID NO: 31 - DNA, 1395 bp, Artificial Sequence
  21R79 Heavy chain
atgaagcacctatggttctttctattattagtggccgctccccgttgggtgttatcgcaggttcagctagttcagtctggagcggaagttaagaaacctggagcatccgtgaaaataagttgcaaggcatccggttactcgttcaccgcatactatatccactgggttaaacaggcaccaggacagggacttgaatggatcggatatatcgctaattataatagagctacaaactataaccaaaaattcaaaggacgcgtgactttcacaactgacacctcaacctcgacagcatacatggaattacggtccctacggtctgacgacactgccgtttactattgcgctagagattatgattatgatgttggaatggactattggggccagggaacactggtgacagtgtcttctgcatccactaagggaccatccgtgttccctttggccccttgctctcgttcgacctctgaatcgactgccgctctgggatgcctcgtgaaagattacttccctgagcctgtgaccgtttcctggaactcgggcgccctaacctctggcgtgcacacattccctgccgtgctacagtcttctggcctatactctttatcttcggttgttaccgtaccttcttctaacttcggaacccaaacttacacctgtaacgtagaccacaagccttcgaacaccaaggtggacaagactgttgagcgaaagtgctgcgttgagtgccctccatgtcctgcacctcctgtggctggcccttctgtgttcctgttccctccaaaacctaaggacactctaatgatctctcggactcctgaggtgacttgcgtggttgtggacgtgtcccacgaggaccctgaggtgcagttcaattggtacgtggacggagtcgaggtgcacaatgcaaagaccaagcctcgggaggaacagttcaactccaccttccgggtggtttctgtgttgaccgttgtgcaccaagactggctgaacggcaaagaatacaagtgcaaggtgtccaacaagggcctgcctgcccctatcgaaaagaccatcagcaagaccaagggccagcctcgcgagcctcaggtgtacaccctgcctcccagccgggaagaaatgaccaagaaccaggtgtccctgacctgtctggtggagggcttctacccttccgacatcgccgttgagtgggagtctaacggacagccggagaacaactacaagactacgcctccaatgctggactccgacggctccttcttcctgtactccgaactgaccgtggacaagtcccggtggcagcagggcaacgtgttctcatgctccgtaatgcacgaagccttgcacaatcactacactcaaaagtccctatccttatctcctggcaagtag

SEQ ID NO: 32 - DNA, 1401 bp, Artificial Sequence
  219R45 Heavy chain
atgaagcatctgtggtttttcctgttgctcgtggcggcacccagatgggtgttgtcccaagtgcagctggtccagagcggggctgaggtgaagaaacccggagcaagcgtaaaagtatcgtgtaaggcctcggggtacacgtttacaaactactggatgcattgggtgcggcaggctccgggacaggggttggaatggatgggtgacattaacccctcaaatggcagaacatcatataaggaaaagttcaaacgccgcgtcacactctccgtggacaagtcaagctcgactgcgtacatggaactttcgtcgctgaggtcggaggacacggcagtgtacttttgcaccatccattatgatgacaagtattaccctctgatggattattggggtcagggtacgttggtcaccgtctccagcgcgtcgacgaaaggtccctcggtatttcccctcgccccctgctcgaggtcgacatccgaatcaacagctgccctcggctgcctggtcaaagactacttcccagagccggtaacggtgtcgtggaactcgggagcgcttacgtccggagtccacacatttccggcggtactgcaatcctcgggactgtattcgttgtcgtcagtggtgactgtcccgtcctccaatttcgggactcagacctatacgtgcaacgtcgaccacaaaccctcaaacaccaaggtggataagacagtggagcgcaagtgctgcgtggagtgtcccccgtgtccggcaccccctgtcgccggaccctcagtctttttgtttccgccgaagcccaaagatacactcatgatctcaagaacgcccgaggtaacatgcgtggtggtcgatgtaagccacgaggatccagaagtacaattcaattggtatgtagacggggtcgaggtccataacgcaaagacgaaaccgagggaagagcagttcaattcgactttccgggtggtgtcggtgcttacagtcgtacatcaggactggttgaacgggaaggagtacaagtgtaaagtatcgaataagggccttccagcgccgattgaaaagaccatctccaagaccaaaggacagccacgagagccgcaagtctatacgcttcctcccagccgagaaaagatgactaaaaaccaggtatcgcttacgtgtctcgtcaagggtttctacccttcggacatcgcggtggaatgggagagcaatggacaaccggaaaacaactacaagacgacaccgcctatgttgaaaagcgatggatcgtttttcctctattcgaaactcacggtcgataagtcacggtggcagcaggggaatgtgttctcctgttcagtgatgcacgaggcgctccacaatcactatacccagaaaagcctgtcactttccccgggaaaatga

SEQ ID NO: 33 - DNA, 1401 bp, Artificial Sequence
  219R45 Heavy chain
atgaagcacctctggttcttcctgctcctcgtggctgctcctcggtgggtcctctcccaagtgcagctggtccagagcggggctgaggtgaagaaacccggagcttccgtcaaagtctcctgtaaggcttccggatacacctttaccaactattggatgcactgggtgcggcaggctcctggacaagggctggaatggatgggagacatcaatccttccaatggcagaacctcctacaaggaaaaattcaaacggcgggtcacactctccgtggacaagtctagctccacagcttacatggaactctcctccctgcggtccgaagacacagctgtctacttctgcaccatccactacgacgacaagtactaccctctgatggactactggggccagggaaccctggtcaccgtgtccagcgcttccacaaaaggaccctccgtctttcccctcgccccctgctcccggtccacatccgaatcaacagctgccctcggctgcctggtcaaagactacttcccagagcctgtcacagtgtcctggaactccggagctctcacatccggagtccacacatttcctgctgtgctccaatcctccggactgtattccctctcctccgtggtgacagtgccttcctccaatttcgggacacagacctatacatgcaacgtggaccacaaaccctccaacaccaaagtcgataagacagtggagcgcaagtgctgcgtggagtgtcccccttgtcctgctccccctgtggctggaccttccgtctttctgtttcctcctaaacctaaagacaccctcatgatctcccggacccccgaggtcacatgcgtggtcgtcgatgtgagccacgaggaccccgaagtccaatttaattggtatgtggacggggtggaggtccataacgctaagaccaaacctagggaagagcagttcaattccactttccgggtggtgtccgtgctgaccgtcgttcatcaggactggctcaacgggaaagaatacaaatgcaaagtctctaataagggcctccctgctcctattgaaaaaacaatttccaaaacaaaaggacaacctcgggagcctcaagtctacacactgccaccttcccgggaaaaaatgacaaaaaatcaagtctccctcacatgtctcgtcaagggattctacccttccgacattgctgtggaatgggaatccaatggacaacctgaaaacaactacaagacaacacctcctatgctcaaaagcgatgggtcctttttcctctattccaaactcacagtcgataagtctcggtggcagcaggggaatgtgttctcctgttccgtgatgcacgaggctctccacaatcactatacccagaaaagcctgtccctctcccctggaaaatga

SEQ ID NO: 34 - DNA, 717 bp, Artificial Sequence
  Light chain
atggtgctgcagacccaggtgttcatctccctgctgctgtggatctccggcgcctacggcgacatcgtgatgacccagtccccagactccctggctgtgtctctgggagagcgggccaccatctcttgcagagcctccgagtccgtggacaactacggcatctccttcatgaagtggttccagcagaagcccggccagcccccaaagctgctgatctacgccgcctccaaccagggatctggcgtgcccgaccggttctctggatccggctctggcaccgactttaccctgaccatcagctccctgcaggccgaggacgtggccgtgtactactgccagcagtccaaagaggtgccctggaccttcggcggaggcaccaaggtggaaatcaagcggaccgtggccgctccctccgtgttcatcttcccaccctccgacgagcagctgaagtccggaaccgcctccgtcgtgtgcctgctgaacaacttctacccccgcgaggccaaggtgcagtggaaggtggacaacgccctgcagtccggcaactcccaggaatccgtcaccgagcaggactccaaggacagcacctactccctgtcctccaccctgaccctgtccaaggccgactacgagaagcacaaggtgtacgcctgcgaagtgacccaccagggcctgtccagccccgtgaccaagtccttcaaccggggcgagtgttag

SEQ ID NO: 35 - DNA, 357 bp, Artificial Sequence
  21M18 Heavy chain variable region
caggtgcagctggtgcagtctggcgccgaagtgaagaaacctggcgcctccgtgaagatctcctgcaaggcctccggctactccttcaccgcttactacatccactgggtcaagcaggcccctgggcagggcctggaatggatcggctacatctcctcctacaacggcgccaccaactacaaccagaaattcaagggccgcgtgaccttcaccaccgacacctccacctccaccgcctacatggaactgcggtccctgcggagcgacgacaccgccgtgtactactgcgccagagactacgactacgacgtgggcatggactactggggccagggcaccctggtcaccgtgtcctct

SEQ ID NO: 36 - DNA, 357 bp, Artificial Sequence
  21R79 Heavy chain variable region
caggtgcagctggtgcagtctggcgccgaagtgaagaaacctggcgcctccgtgaagatctcctgcaaggcctccggctactccttcaccgcctactacatccactgggtgaaacaggcaccaggccagggactggaatggatcggctatatcgccaactacaaccgggccaccaactacaaccagaaattcaagggccgcgtgaccttcaccaccgacacctccacctccacagcctacatggaactgcggtccctgcggagcgacgacaccgccgtgtactactgcgccagagactacgactacgacgtgggcatggactactggggccagggcaccctggtgacagtgtcctcc

SEQ ID NO: 37 - DNA, 357 bp, Artificial Sequence
  21R79 Heavy chain variable region
caggttcagctagttcagtctggagcggaagttaagaaacctggagcatccgtgaaaataagttgcaaggcatccggttactcgttcaccgcatactatatccactgggttaaacaggcaccaggacagggacttgaatggatcggatatatcgctaattataatagagctacaaactataaccaaaaattcaaaggacgcgtgactttcacaactgacacctcaacctcgacagcatacatggaattacggtccctacggtctgacgacactgccgtttactattgcgctagagattatgattatgatgttggaatggactattggggccagggaacactggtgacagtgtcttct

SEQ ID NO: 38 - DNA, 360 bp, Artificial Sequence
  219R45 Heavy chain variable region
caagtgcagctggtccagagcggggctgaggtgaagaaacccggagcaagcgtaaaagtatcgtgtaaggcctcggggtacacgtttacaaactactggatgcattgggtgcggcaggctccgggacaggggttggaatggatgggtgacattaacccctcaaatggcagaacatcatataaggaaaagttcaaacgccgcgtcacactctccgtggacaagtcaagctcgactgcgtacatggaactttcgtcgctgaggtcggaggacacggcagtgtacttttgcaccatccattatgatgacaagtattaccctctgatggattattggggtcagggtacgttggtcaccgtctcc

SEQ ID NO: 39 - DNA, 363 bp, Artificial Sequence
  219R45 Heavy chain variable region
caagtgcagctggtccagagcggggctgaggtgaagaaacccggagcttccgtcaaagtctcctgtaaggcttccggatacacctttaccaactattggatgcactgggtgcggcaggctcctggacaagggctggaatggatgggagacatcaatccttccaatggcagaacctcctacaaggaaaaattcaaacggcgggtcacactctccgtggacaagtctagctccacagcttacatggaactctcctccctgcggtccgaagacacagctgtctacttctgcaccatccactacgacgacaagtactaccctctgatggactactggggccagggaaccctggtcaccgtgtccagc

SEQ ID NO: 40 - DNA, 333 bp, Artificial Sequence
  Light chain variable region
gacatcgtgatgacccagtccccagactccctggctgtgtctctgggagagcgggccaccatctcttgcagagcctccgagtccgtggacaactacggcatctccttcatgaagtggttccagcagaagcccggccagcccccaaagctgctgatctacgccgcctccaaccagggatctggcgtgcccgaccggttctctggatccggctctggcaccgactttaccctgaccatcagctccctgcaggccgaggacgtggccgtgtactactgccagcagtccaaagaggtgccctggaccttcggcggaggcaccaaggtggaaatcaag

SEQ ID NO: 41 - protein, 330 aa, Homo sapiens [sequence omitted]

SEQ ID NO: 42 - protein, 326 aa, Homo sapiens
ASTKGPSVFPLAPCSRSTSESTAALGCLVKDYFPEPVTVSWNSGALTSGVHTFPAVLQSSGLYSLSSVVTVPSSNFGTQTYTCNVDHKPSNTKVDKTVERKCCVECPPCPAPPVAGPSVFLFPPKPKDTLMISRTPEVTCVVVDVSHEDPEVQFNWYVDGVEVHNAKTKPREEQFNSTFRVVSVLTVVHQDWLNGKEYKCKVSNKGLPAPIEKTISKTKGQPREPQVYTLPPSREEMTKNQVSLTCLVKGFYPSDIAVEWESNGQPENNYKTTPPMLDSDGSFFLYSKLTVDKSRWQQGNVFSCSVMHEALHNHYTQKSLSLSPGK

SEQ ID NO: 43 - protein, 377 aa, Homo sapiens
ASTKGPSVFPLAPCSRSTSGGTAALGCLVKDYFPEPVTVSWNSGALTSGVHTFPAVLQSSGLYSLSSVVTVPSSSLGTQTYTCNVNHKPSNTKVDKRVELKTPLGDTTHTCPRCPEPKSCDTPPPCPRCPEPKSCDTPPPCPRCPEPKSCDTPPPCPRCPAPELLGGPSVFLFPPKPKDTLMISRTPEVTCVVVDVSHEDPEVQFKWYVDGVEVHNAKTKPREEQYNSTFRVVSVLTVLHQDWLNGKEYKCKVSNKALPAPIEKTISKTKGQPREPQVYTLPPSREEMTKNQVSLTCLVKGFYPSDIAVEWESSGQPENNYNTTPPMLDSDGSFFLYSKLTVDKSRWQQGNIFSCSVMHEALHNRFTQKSLSLSPGK

SEQ ID NO: 44 - protein, 327 aa, Homo sapiens
ASTKGPSVFPLAPCSRSTSESTAALGCLVKDYFPEPVTVSWNSGALTSGVHTFPAVLQSSGLYSLSSVVTVPSSSLGTKTYTCNVDHKPSNTKVDKRVESKYGPPCPSCPAPEFLGGPSVFLFPPKPKDTLMISRTPEVTCVVVDVSQEDPEVQFNWYVDGVEVHNAKTKPREEQFNSTYRVVSVLTVLHQDWLNGKEYKCKVSNKGLPSSIEKTISKAKGQPREPQVYTLPPSQEEMTKNQVSLTCLVKGFYPSDIAVEWESNGQPENNYKTTPPVLDSDGSFFLYSRLTVDKSRWQEGNVFSCSVMHEALHNHYTQKSLSLSLGK

SEQ ID NO: 45 - protein, 8 aa, Artificial Sequence
  FLAG peptide
DYKDDDDK

SEQ ID NO: 46 - protein, 464 aa, Artificial Sequence
  Parental 21R79 Heavy chain
  SIGNAL (1)..(19)
MKHLWFFLLLVAAPRWVLSQVQLVQSGAEVKKPGASVKISCKASGYSFTAYYIHWVKQAPGQGLEWIGYIANYNRATNYNQKFKGRVTFTTDTSTSTAYMELRSLRSDDTAVYYCARDYDYDVGMDYWGQGTLVTVSSASTKGPSVFPLAPCSRSTSESTAALGCLVKDYFPEPVTVSWNSGALTSGVHTFPAVLQSSGLYSLSSVVTVPSSNFGTQTYTCNVDHKPSNTKVDKTVERKCCVECPPCPAPPVAGPSVFLFPPKPKDTLMISRTPEVTCVVVDVSHEDPEVQFNWYVDGVEVHNAKTKPREEQFNSTFRVVSVLTVVHQDWLNGKEYKCKVSNKGLPAPIEKTISKTKGQPREPQVYTLPPSREEMTKNQVSLTCLVKGFYPSDIAVEWESNGQPENNYKTTPPMLDSDGSFFLYSKLTVDKSRWQQGNVFSCSVMHEALHNHYTQKSLSLSPGK

SEQ ID NO: 47 - protein, 466 aa, Artificial Sequence
  Parental 219R45 Heavy chain
  SIGNAL (1)..(19)
MKHLWFFLLLVAAPRWVLSQVQLVQSGAEVKKPGASVKVSCKASGYTFTNYWMHWVRQAPGQGLEWMGDINPSNGRTSYKEKFKRRVTLSVDKSSSTAYMELSSLRSEDTAVYFCTIHYDDKYYPLMDYWGQGTLVTVSSASTKGPSVFPLAPCSRSTSESTAALGCLVKDYFPEPVTVSWNSGALTSGVHTFPAVLQSSGLYSLSSVVTVPSSNFGTQTYTCNVDHKPSNTKVDKTVERKCCVECPPCPAPPVAGPSVFLFPPKPKDTLMISRTPEVTCVVVDVSHEDPEVQFNWYVDGVEVHNAKTKPREEQFNSTFRVVSVLTVVHQDWLNGKEYKCKVSNKGLPAPIEKTISKTKGQPREPQVYTLPPSREEMTKNQVSLTCLVKGFYPSDIAVEWESNGQPENNYKTTPPMLDSDGSFFLYSKLTVDKSRWQQGNVFSCSVMHEALHNHYTQKSLSLSPGK

SEQ ID NO: 48 - protein, 445 aa, Artificial Sequence
  Parental 21R79 Heavy chain
QVQLVQSGAEVKKPGASVKISCKASGYSFTAYYIHWVKQAPGQGLEWIGYIANYNRATNYNQKFKGRVTFTTDTSTSTAYMELRSLRSDDTAVYYCARDYDYDVGMDYWGQGTLVTVSSASTKGPSVFPLAPCSRSTSESTAALGCLVKDYFPEPVTVSWNSGALTSGVHTFPAVLQSSGLYSLSSVVTVPSSNFGTQTYTCNVDHKPSNTKVDKTVERKCCVECPPCPAPPVAGPSVFLFPPKPKDTLMISRTPEVTCVVVDVSHEDPEVQFNWYVDGVEVHNAKTKPREEQFNSTFRVVSVLTVVHQDWLNGKEYKCKVSNKGLPAPIEKTISKTKGQPREPQVYTLPPSREEMTKNQVSLTCLVKGFYPSDIAVEWESNGQPENNYKTTPPMLDSDGSFFLYSKLTVDKSRWQQGNVFSCSVMHEALHNHYTQKSLSLSPGK

SEQ ID NO: 49 - protein, 447 aa, Artificial Sequence
  Parental 219R45 Heavy chain
QVQLVQSGAEVKKPGASVKVSCKASGYTFTNYWMHWVRQAPGQGLEWMGDINPSNGRTSYKEKFKRRVTLSVDKSSSTAYMELSSLRSEDTAVYFCTIHYDDKYYPLMDYWGQGTLVTVSSASTKGPSVFPLAPCSRSTSESTAALGCLVKDYFPEPVTVSWNSGALTSGVHTFPAVLQSSGLYSLSSVVTVPSSNFGTQTYTCNVDHKPSNTKVDKTVERKCCVECPPCPAPPVAGPSVFLFPPKPKDTLMISRTPEVTCVVVDVSHEDPEVQFNWYVDGVEVHNAKTKPREEQFNSTFRVVSVLTVVHQDWLNGKEYKCKVSNKGLPAPIEKTISKTKGQPREPQVYTLPPSREEMTKNQVSLTCLVKGFYPSDIAVEWESNGQPENNYKTTPPMLDSDGSFFLYSKLTVDKSRWQQGNVFSCSVMHEALHNHYTQKSLSLSPGK

SEQ ID NO: 50 - DNA, 357 bp, Artificial Sequence
  Parental 21R79 Heavy chain variable region
caagtgcagctcgtgcagtcaggggcggaggtcaagaagccgggagcatcggtcaaaatctcgtgtaaggcctcggggtactcctttactgcgtattacatccattgggtaaagcaggcgccagggcagggattggagtggattgggtatatcgccaattacaatcgcgcgacgaactataaccagaaattcaagggaagggtgaccttcacaacggatacatcgacatcgacggcctacatggaacttcgcagcctgcgatcagatgacacggcggtatactattgcgcaagagattacgactatgatgtgggaatggactattggggtcaaggtactctggtcacagtctcctcc

SEQ ID NO: 51 - DNA, 363 bp, Artificial Sequence
  Parental 219R45 Heavy chain variable region
caggtacagctcgtgcaatcgggggcagaggtcaaaaagcccggtgcgtcggtaaaggtcagctgcaaagcgtcaggttatacattcacgaattactggatgcattgggtcagacaggcccctggacaagggcttgaatggatgggagatatcaatccgtcgaacggacggactagctataaggagaagtttaagaggcgcgtaacactgtcggtggacaaatcgtcctcaacggcctacatggagttgtcatccctgcggtcggaagatacggcggtctacttctgtactatccactatgacgataagtactacccgcttatggactactggggtcagggaacattggtaaccgtgagcagc

SEQ ID NO: 52 - DNA, 1392 bp, Artificial Sequence
  Parental 21R79 Heavy chain
atgaaacacttgtggtttttcctcttgctcgtggcagctcctcggtgggtactttcacaagtgcagctcgtgcagtcaggggcggaggtcaagaagccgggagcatcggtcaaaatctcgtgtaaggcctcggggtactcctttactgcgtattacatccattgggtaaagcaggcgccagggcagggattggagtggattgggtatatcgccaattacaatcgcgcgacgaactataaccagaaattcaagggaagggtgaccttcacaacggatacatcgacatcgacggcctacatggaacttcgcagcctgcgatcagatgacacggcggtatactattgcgcaagagattacgactatgatgtgggaatggactattggggtcaaggtactctggtcacagtctcctccgccagcaccaagggccctagcgtcttccctctggctccctgcagcaggagcaccagcgagagcacagccgccctgggctgcctggtcaaggactacttccccgaaccggtgacggtgtcgtggaactcaggcgctctgaccagcggcgtgcacaccttcccagctgtcctacagtcctcaggactctactccctcagcagcgtggtgaccgtgccctccagcaacttcggcacccagacctacacctgcaacgtagatcacaagcccagcaacaccaaggtggacaagacagttgagcgcaaatgttgtgtcgagtgcccaccgtgcccagcaccacctgtggcaggaccgtcagtcttcctcttccccccaaaacccaaggacaccctcatgatctcccggacccctgaggtcacgtgcgtggtggtggacgtgagccacgaagaccccgaggtccagttcaactggtacgtggacggcgtggaggtgcataatgccaagacaaagccacgggaggagcagttcaacagcacgttccgtgtggtcagcgtcctcaccgttgtgcaccaggactggctgaacggcaaggagtacaagtgcaaggtctccaacaaaggcctcccagcccccatcgagaaaaccatctccaaaaccaaagggcagccccgagaaccacaggtgtacaccctgcccccatcccgggaggagatgaccaagaaccaggtcagcctgacctgcctggtcaaaggcttctaccccagcgacatcgccgtggagtgggagagcaatgggcagccggagaacaactacaagaccacacctcccatgctggactccgacggctccttcttcctctacagcaagctcaccgtggacaagagcaggtggcagcaggggaacgtcttctcatgctccgtgatgcatgaggctctgcacaaccactacacgcagaagagcctctccctgtctccgggtaaa

SEQ ID NO: 53 - DNA, 1398 bp, Artificial Sequence
  Parental 219R45 Heavy chain
atgaaacacctctggttctttttgctcctggtggcagctccccgatgggtgcttagccaggtacagctcgtgcaatcgggggcagaggtcaaaaagcccggtgcgtcggtaaaggtcagctgcaaagcgtcaggttatacattcacgaattactggatgcattgggtcagacaggcccctggacaagggcttgaatggatgggagatatcaatccgtcgaacggacggactagctataaggagaagtttaagaggcgcgtaacactgtcggtggacaaatcgtcctcaacggcctacatggagttgtcatccctgcggtcggaagatacggcggtctacttctgtactatccactatgacgataagtactacccgcttatggactactggggtcagggaacattggtaaccgtgagcagcgcgtccacaaagggccctagcgtcttccctctggctccctgcagcaggagcaccagcgagagcacagccgccctgggctgcctggtcaaggactacttccccgaaccggtgacggtgtcgtggaactcaggcgctctgaccagcggcgtgcacaccttcccagctgtcctacagtcctcaggactctactccctcagcagcgtggtgaccgtgccctccagcaacttcggcacccagacctacacctgcaacgtagatcacaagcccagcaacaccaaggtggacaagacagttgagcgcaaatgttgtgtcgagtgcccaccgtgcccagcaccacctgtggcaggaccgtcagtcttcctcttccccccaaaacccaaggacaccctcatgatctcccggacccctgaggtcacgtgcgtggtggtggacgtgagccacgaagaccccgaggtccagttcaactggtacgtggacggcgtggaggtgcataatgccaagacaaagccacgggaggagcagttcaacagcacgttccgtgtggtcagcgtcctcaccgttgtgcaccaggactggctgaacggcaaggagtacaagtgcaaggtctccaacaaaggcctcccagcccccatcgagaaaaccatctccaaaaccaaagggcagccccgagaaccacaggtgtacaccctgcccccatcccgggaggagatgaccaagaaccaggtcagcctgacctgcctggtcaaaggcttctaccccagcgacatcgccgtggagtgggagagcaatgggcagccggagaacaactacaagaccacacctcccatgctggactccgacggctccttcttcctctacagcaagctcaccgtggacaagagcaggtggcagcaggggaacgtcttctcatgctccgtgatgcatgaggctctgcacaaccactacacgcagaagagcctctccctgtctccgggtaaa

SEQ ID NO: 54 - DNA, 333 bp, Artificial Sequence
  Parental 21R79 and 219R45 light chain variable region
gacatcgtgatgacccagtcccctgactccctggctgtgtccctgggcgagagggccaccatctcctgcagagccagcgaatccgtcgataattatggcatttcctttatgaagtggttccagcagaaaccaggacagcctcctaagctgctcatttacgctgcatccaaccaagggtccggggtccctgacaggttctccggcagcgggtccggaacagatttcactctcaccatcagcagcctgcaggctgaagatgtggctgtctattactgtcagcaaagcaaggaggtgccttggacattcggaggagggaccaaggtggaaatcaaa

SEQ ID NO: 55 - DNA, 717 bp, Artificial Sequence
  Parental 21R79 and 219R45 light chain
atggtgctccagacccaggtcttcatttccctgctgctctggatcagcggagcctacggggacatcgtgatgacccagtcccctgactccctggctgtgtccctgggcgagagggccaccatctcctgcagagccagcgaatccgtcgataattatggcatttcctttatgaagtggttccagcagaaaccaggacagcctcctaagctgctcatttacgctgcatccaaccaagggtccggggtccctgacaggttctccggcagcgggtccggaacagatttcactctcaccatcagcagcctgcaggctgaagatgtggctgtctattactgtcagcaaagcaaggaggtgccttggacattcggaggagggaccaaggtggaaatcaaacgtacggtggctgccccctccgtcttcatcttcccccccagcgatgagcagctgaaaagcggcactgccagcgtggtgtgcctgctgaataacttctatccccgggaggccaaagtgcagtggaaggtggataacgccctccaaagcggcaactcccaggagagcgtcacagagcaggacagcaaggacagcacctacagcctcagcagcaccctgaccctgagcaaagccgactacgagaaacacaaagtctacgcctgcgaagtcacccatcagggcctgagcagccccgtcacaaagagcttcaacaggggcgagtgttga

SEQ ID NO: 56 - protein, 445 aa, Artificial Sequence
  21R75 Heavy chain
QVQLVQSGAEVKKPGASVKISCKASGYSFTAYYIHWVKQAPGQGLEWIGYIAGYKDATNYNQKFKGRVTFTTDTSTSTAYMELRSLRSDDTAVYYCARDYDYDVGMDYWGQGTLVTVSSASTKGPSVFPLAPCSRSTSESTAALGCLVKDYFPEPVTVSWNSGALTSGVHTFPAVLQSSGLYSLSSVVTVPSSNFGTQTYTCNVDHKPSNTKVDKTVERKCCVECPPCPAPPVAGPSVFLFPPKPKDTLMISRTPEVTCVVVDVSHEDPEVQFNWYVDGVEVHNAKTKPREEQFNSTFRVVSVLTVVHQDWLNGKEYKCKVSNKGLPAPIEKTISKTKGQPREPQVYTLPPSREEMTKNQVSLTCLVEGFYPSDIAVEWESNGQPENNYKTTPPMLDSDGSFFLYSELTVDKSRWQQGNVFSCSVMHEALHNHYTQKSLSLSPGK

SEQ ID NO: 57 - protein, 464 aa, Artificial Sequence
  21R75 Heavy chain
  SIGNAL (1)..(19)
MKHLWFFLLLVAAPRWVLSQVQLVQSGAEVKKPGASVKISCKASGYSFTAYYIHWVKQAPGQGLEWIGYIAGYKDATNYNQKFKGRVTFTTDTSTSTAYMELRSLRSDDTAVYYCARDYDYDVGMDYWGQGTLVTVSSASTKGPSVFPLAPCSRSTSESTAALGCLVKDYFPEPVTVSWNSGALTSGVHTFPAVLQSSGLYSLSSVVTVPSSNFGTQTYTCNVDHKPSNTKVDKTVERKCCVECPPCPAPPVAGPSVFLFPPKPKDTLMISRTPEVTCVVVDVSHEDPEVQFNWYVDGVEVHNAKTKPREEQFNSTFRVVSVLTVVHQDWLNGKEYKCKVSNKGLPAPIEKTISKTKGQPREPQVYTLPPSREEMTKNQVSLTCLVEGFYPSDIAVEWESNGQPENNYKTTPPMLDSDGSFFLYSELTVDKSRWQQGNVFSCSVMHEALHNHYTQKSLSLSPGK

SEQ ID NO: 58 - protein, 119 aa, Artificial Sequence
  21R75 Heavy chain variable region
QVQLVQSGAEVKKPGASVKISCKASGYSFTAYYIHWVKQAPGQGLEWIGYIAGYKDATNYNQKFKGRVTFTTDTSTSTAYMELRSLRSDDTAVYYCARDYDYDVGMDYWGQGTLVTVSS

SEQ ID NO: 59 - protein, 17 aa, Artificial Sequence
  21R75 Heavy chain CDR2
YIAGYKDATNYNQKFKG

SEQ ID NO: 60 - DNA, 1392 bp, Artificial Sequence
  21R75 Heavy chain
  sig_peptide (1)..(57)
atgaagcacctgtggttctttctgctgctggtggccgctcccagatgggtgctgtcccaggtgcagctggtgcagtctggcgccgaagtgaagaaacctggcgcctccgtgaagatctcctgcaaggcctccggctactccttcaccgcctactacatccactgggtcaagcaggcccctggacagggcctggaatggatcggctatatcgccggctacaaggacgccaccaactacaaccagaaattcaagggcagagtgaccttcaccaccgacacctccacctctaccgcctacatggaactgcggtccctgcggagcgacgacaccgccgtgtactactgcgccagagactacgactacgacgtgggcatggactactggggccagggcacactcgtgaccgtgtcctctgcttccaccaagggcccctccgtgtttcctctggccccttgctccagatccacctccgagtctaccgccgctctgggctgcctcgtgaaggactacttccccgagcccgtgacagtgtcttggaactctggcgccctgacctccggcgtgcacacctttccagctgtgctgcagtcctccggcctgtactccctgtcctccgtcgtgactgtgccctcctccaacttcggcacccagacctacacctgtaacgtggaccacaagccctccaacaccaaggtggacaagaccgtggaacggaagtgctgcgtggaatgccccccttgtcctgcccctcctgtggctggccctagcgtgttcctgttccccccaaagcccaaggacaccctgatgatctcccggacccccgaagtgacctgcgtggtggtggatgtgtcccacgaggaccccgaggtgcagttcaattggtacgtggacggcgtggaagtgcacaacgccaagaccaagcccagagaggaacagttcaactccaccttccgggtggtgtccgtgctgaccgtggtgcatcaggactggctgaacggcaaagagtacaagtgcaaggtgtccaacaagggcctgcctgcccccatcgaaaagaccatctctaagaccaagggacagccccgcgagccccaggtgtacacactgcctccatcccgggaagagatgaccaagaaccaggtgtccctgacctgtctggtggaaggcttctacccctccgatatcgccgtggaatgggagtccaacggccagcccgagaacaactacaagaccaccccccccatgctggactccgacggctcattcttcctgtacagcgagctgacagtggacaagtcccggtggcagcagggcaacgtgttctcctgctccgtgatgcacgaggccctgcacaaccactacacccagaagtccctgtccctgagccccggcaag

SEQ ID NO: 61 - DNA, 1392 bp, Artificial Sequence
  21R75 Heavy chain
  sig_peptide (1)..(57)
atgaagcacctgtggttctttctgctgctggtggccgctcccagatgggtgctgtcccaggttcagctagttcagtctggagcggaagttaagaaacctggagcatccgtgaaaataagttgcaaggcatccggttactcgttcaccgcatactatatccactgggttaaacaggcaccaggacagggacttgaatggatcggatatatcgctggatataaagatgctacaaactataaccaaaaattcaaaggacgcgtgactttcacaactgacacctcaacctcgacagcatacatggaattacggtccctacggtctgacgacactgccgtttactattgcgctagagattatgattatgatgttggaatggactattggggccagggaacactggtgacagtgtcttctgcatccactaagggaccatccgtgttccctttggccccttgctctcgttcgacctctgaatcgactgccgctctgggatgcctcgtgaaagattacttccctgagcctgtgaccgtttcctggaactcgggcgccctaacctctggcgtgcacacattccctgccgtgctacagtcttctggcctatactctttatcttcggttgttaccgtaccttcttctaacttcggaacccaaacttacacctgtaacgtagaccacaagccttcgaacaccaaggtggacaagactgttgagcgaaagtgctgcgttgagtgccctccatgtcctgcacctcctgtggctggcccttctgtgttcctgttccctccaaaacctaaggacactctaatgatctctcggactcctgaggtgacttgcgtggttgtggacgtgtcccacgaggaccctgaggtgcagttcaattggtacgtggacggagtcgaggtgcacaatgcaaagaccaagcctcgggaggaacagttcaactccaccttccgggtggtttctgtgttgaccgttgtgcaccaagactggctgaacggcaaagaatacaagtgcaaggtgtccaacaagggcctgcctgcccctatcgaaaagaccatcagcaagaccaagggccagcctcgcgagcctcaggtgtacaccctgcctcccagccgggaagaaatgaccaagaaccaggtgtccctgacctgtctggtggagggcttctacccttccgacatcgccgttgagtgggagtctaacggacagccggagaacaactacaagactacgcctccaatgctggactccgacggctccttcttcctgtactccgaactgaccgtggacaagtcccggtggcagcagggcaacgtgttctcatgctccgtaatgcacgaagccttgcacaatcactacactcaaaagtccctatccttatctcctggcaag

SEQ ID NO: 62 - protein, 445 aa, Artificial Sequence
  21R83 Heavy chain
QVQLVQSGAEVKKPGASVKISCKASGYSFTAYYIHWVKQAPGQGLEWIGYISNYNRATNYNQKFKGRVTFTTDTSTSTAYMELRSLRSDDTAVYYCARDYDYDVGMDYWGQGTLVTVSSASTKGPSVFPLAPCSRSTSESTAALGCLVKDYFPEPVTVSWNSGALTSGVHTFPAVLQSSGLYSLSSVVTVPSSNFGTQTYTCNVDHKPSNTKVDKTVERKCCVECPPCPAPPVAGPSVFLFPPKPKDTLMISRTPEVTCVVVDVSHEDPEVQFNWYVDGVEVHNAKTKPREEQFNSTFRVVSVLTVVHQDWLNGKEYKCKVSNKGLPAPIEKTISKTKGQPREPQVYTLPPSREEMTKNQVSLTCLVEGFYPSDIAVEWESNGQPENNYKTTPPMLDSDGSFFLYSELTVDKSRWQQGNVFSCSVMHEALHNHYTQKSLSLSPGK

SEQ ID NO: 63 - protein, 464 aa, Artificial Sequence
  21R83 Heavy chain
  SIGNAL (1)..(19)
MKHLWFFLLLVAAPRWVLSQVQLVQSGAEVKKPGASVKISCKASGYSFTAYYIHWVKQAPGQGLEWIGYISNYNRATNYNQKFKGRVTFTTDTSTSTAYMELRSLRSDDTAVYYCARDYDYDVGMDYWGQGTLVTVSSASTKGPSVFPLAPCSRSTSESTAALGCLVKDYFPEPVTVSWNSGALTSGVHTFPAVLQSSGLYSLSSVVTVPSSNFGTQTYTCNVDHKPSNTKVDKTVERKCCVECPPCPAPPVAGPSVFLFPPKPKDTLMISRTPEVTCVVVDVSHEDPEVQFNWYVDGVEVHNAKTKPREEQFNSTFRVVSVLTVVHQDWLNGKEYKCKVSNKGLPAPIEKTISKTKGQPREPQVYTLPPSREEMTKNQVSLTCLVEGFYPSDIAVEWESNGQPENNYKTTPPMLDSDGSFFLYSELTVDKSRWQQGNVFSCSVMHEALHNHYTQKSLSLSPGK

SEQ ID NO: 64 - protein, 119 aa, Artificial Sequence
  21R83 Heavy chain variable region
QVQLVQSGAEVKKPGASVKISCKASGYSFTAYYIHWVKQAPGQGLEWIGYISNYNRATNYNQKFKGRVTFTTDTSTSTAYMELRSLRSDDTAVYYCARDYDYDVGMDYWGQGTLVTVSS

SEQ ID NO: 65 - protein, 17 aa, Artificial Sequence
  21R83 Heavy chain CDR2
YISNYNRATNYNQKFKG

SEQ ID NO: 66 - DNA, 1392 bp, Artificial Sequence
  21R83 Heavy chain
  sig_peptide (1)..(57)
atgaagcacctgtggttctttctgctgctggtggccgctcccagatgggtgctgtcccaggtgcagctggtgcagtctggcgccgaagtgaagaaacctggcgcctccgtgaagatctcctgcaaggcctccggctactccttcaccgcctactacatccactgggtcaagcaggcccctggacagggcctggaatggatcggctacatctccaactacaaccgggccaccaattacaaccagaaattcaagggccgcgtgaccttcaccaccgacacctctacctctaccgcctacatggaactgcggtccctgcggagcgacgacaccgccgtgtactactgcgccagagactacgactacgacgtgggcatggactactggggccagggcacactcgtgaccgtgtctagcgcttccaccaagggcccctccgtgtttcctctggccccttgctccagatccacctccgagtctaccgccgctctgggctgcctcgtgaaggactacttccccgagcccgtgacagtgtcctggaactctggcgctctgacctccggcgtgcacacctttccagctgtgctgcagtcctccggcctgtactccctgtcctccgtcgtgactgtgccctcctccaacttcggcacccagacctacacctgtaacgtggaccacaagccctccaacaccaaggtggacaagaccgtggaacggaagtgctgcgtggaatgccccccttgtcctgcccctcctgtggctggccctagcgtgttcctgttccccccaaagcccaaggacaccctgatgatctcccggacccccgaagtgacctgcgtggtggtggatgtgtcccacgaggaccccgaggtgcagttcaattggtacgtggacggcgtggaagtgcacaacgccaagaccaagcccagagaggaacagttcaactccaccttccgggtggtgtccgtgctgaccgtggtgcatcaggactggctgaacggcaaagagtacaagtgcaaggtgtccaacaagggcctgcctgcccccatcgaaaagaccatctctaagaccaagggacagccccgcgagccccaggtgtacacactgcctccatcccgggaagagatgaccaagaaccaggtgtccctgacctgtctggtggaaggcttctacccctccgatatcgccgtggaatgggagtccaacggccagcccgagaacaactacaagaccaccccccccatgctggactccgacggctcattcttcctgtacagcgagctgacagtggacaagtcccggtggcagcagggcaacgtgttctcctgctccgtgatgcacgaggccctgcacaaccactacacccagaagtccctgtccctgagccccggcaag

SEQ ID NO: 67 - DNA, 1392 bp, Artificial Sequence; identical to SEQ ID NO: 61
  21R75 Heavy chain
  sig_peptide (1)..(57)

SEQ ID NO: 68 - DNA, 357 bp, Artificial Sequence
  21R75 Heavy chain variable region
caggtgcagctggtgcagtctggcgccgaagtgaagaaacctggcgcctccgtgaagatctcctgcaaggcctccggctactccttcaccgcctactacatccactgggtcaagcaggcccctggacagggcctggaatggatcggctatatcgccggctacaaggacgccaccaactacaaccagaaattcaagggcagagtgaccttcaccaccgacacctccacctctaccgcctacatggaactgcggtccctgcggagcgacgacaccgccgtgtactactgcgccagagactacgactacgacgtgggcatggactactggggccagggcacactcgtgaccgtgtcctct

SEQ ID NO: 69 - DNA, 357 bp, Artificial Sequence
  21R75 Heavy chain variable region
caggttcagctagttcagtctggagcggaagttaagaaacctggagcatccgtgaaaataagttgcaaggcatccggttactcgttcaccgcatactatatccactgggttaaacaggcaccaggacagggacttgaatggatcggatatatcgctggatataaagatgctacaaactataaccaaaaattcaaaggacgcgtgactttcacaactgacacctcaacctcgacagcatacatggaattacggtccctacggtctgacgacactgccgtttactattgcgctagagattatgattatgatgttggaatggactattggggccagggaacactggtgacagtgtcttct

SEQ ID NO: 70 - DNA, 357 bp, Artificial Sequence
  21R83 Heavy chain variable region
caggtgcagctggtgcagtctggcgccgaagtgaagaaacctggcgcctccgtgaagatctcctgcaaggcctccggctactccttcaccgcctactacatccactgggtcaagcaggcccctggacagggcctggaatggatcggctacatctccaactacaaccgggccaccaattacaaccagaaattcaagggccgcgtgaccttcaccaccgacacctctacctctaccgcctacatggaactgcggtccctgcggagcgacgacaccgccgtgtactactgcgccagagactacgactacgacgtgggcatggactactggggccagggcacactcgtgaccgtgtctagc

SEQ ID NO: 71 - DNA, 357 bp, Artificial Sequence; identical to SEQ ID NO: 69
  21R75 Heavy chain variable region

SEQ ID NO: 72 - DNA, 1395 bp, Artificial Sequence
  21R83 Heavy chain
  sig_peptide (1)..(57)
atgaagcacctatggttctttctattattagtggccgctccccgttgggtgttatcgcaggttcagctagttcagtctggagcggaagttaagaaacctggagcatccgtgaaaataagttgcaaggcatccggttactcgttcaccgcatactatatccactgggttaaacaggcaccaggacagggacttgaatggatcggatatatctccaattataatagagctacaaactataaccaaaaattcaaaggacgcgtgactttcacaactgacacctcaacctcgacagcatacatggaattacggtccctacggtctgacgacactgccgtttactattgcgctagagattatgattatgatgttggaatggactattggggccagggaacactggtgacagtgtcttctgcatccactaagggaccatccgtgttccctttggccccttgctctcgttcgacctctgaatcgactgccgctctgggatgcctcgtgaaagattacttccctgagcctgtgaccgtttcctggaactcgggcgccctaacctctggcgtgcacacattccctgccgtgctacagtcttctggcctatactctttatcttcggttgttaccgtaccttcttctaacttcggaacccaaacttacacctgtaacgtagaccacaagccttcgaacaccaaggtggacaagactgttgagcgaaagtgctgcgttgagtgccctccatgtcctgcacctcctgtggctggcccttctgtgttcctgttccctccaaaacctaaggacactctaatgatctctcggactcctgaggtgacttgcgtggttgtggacgtgtcccacgaggaccctgaggtgcagttcaattggtacgtggacggagtcgaggtgcacaatgcaaagaccaagcctcgggaggaacagttcaactccaccttccgggtggtttctgtgttgaccgttgtgcaccaagactggctgaacggcaaagaatacaagtgcaaggtgtccaacaagggcctgcctgcccctatcgaaaagaccatcagcaagaccaagggccagcctcgcgagcctcaggtgtacaccctgcctcccagccgggaagaaatgaccaagaaccaggtgtccctgacctgtctggtggagggcttctacccttccgacatcgccgttgagtgggagtctaacggacagccggagaacaactacaagactacgcctccaatgctggactccgacggctccttcttcctgtactccgaactgaccgtggacaagtcccggtggcagcagggcaacgtgttctcatgctccgtaatgcacgaagccttgcacaatcactacactcaaaagtccctatccttatctcctggcaagtag

SEQ ID NO: 73 - DNA, 357 bp, Artificial Sequence
  21R83 Heavy chain variable region
caggttcagctagttcagtctggagcggaagttaagaaacctggagcatccgtgaaaataagttgcaaggcatccggttactcgttcaccgcatactatatccactgggttaaacaggcaccaggacagggacttgaatggatcggatatatctccaattataatagagctacaaactataaccaaaaattcaaaggacgcgtgactttcacaactgacacctcaacctcgacagcatacatggaattacggtccctacggtctgacgacactgccgtttactattgcgctagagattatgattatgatgttggaatggactattggggccagggaacactggtgacagtgtcttct

SEQ ID NO: 74 - DNA, 1395 bp, Artificial Sequence
  21R75 Heavy chain
  sig_peptide (1)..(57)
atgaagcacctatggttctttctattattagtggccgctccccgttgggtgttatcgcaggttcagctagttcagtctggagcggaagttaagaaacctggagcatccgtgaaaataagttgcaaggcatccggttactcgttcaccgcatactatatccactgggttaaacaggcaccaggacagggacttgaatggatcggatatatcgctggatataaagatgctacaaactataaccaaaaattcaaaggacgcgtgactttcacaactgacacctcaacctcgacagcatacatggaattacggtccctacggtctgacgacactgccgtttactattgcgctagagattatgattatgatgttggaatggactattggggccagggaacactggtgacagtgtcttctgcatccactaagggaccatccgtgttccctttggccccttgctctcgttcgacctctgaatcgactgccgctctgggatgcctcgtgaaagattacttccctgagcctgtgaccgtttcctggaactcgggcgccctaacctctggcgtgcacacattccctgccgtgctacagtcttctggcctatactctttatcttcggttgttaccgtaccttcttctaacttcggaacccaaacttacacctgtaacgtagaccacaagccttcgaacaccaaggtggacaagactgttgagcgaaagtgctgcgttgagtgccctccatgtcctgcacctcctgtggctggcccttctgtgttcctgttccctccaaaacctaaggacactctaatgatctctcggactcctgaggtgacttgcgtggttgtggacgtgtcccacgaggaccctgaggtgcagttcaattggtacgtggacggagtcgaggtgcacaatgcaaagaccaagcctcgggaggaacagttcaactccaccttccgggtggtttctgtgttgaccgttgtgcaccaagactggctgaacggcaaagaatacaagtgcaaggtgtccaacaagggcctgcctgcccctatcgaaaagaccatcagcaagaccaagggccagcctcgcgagcctcaggtgtacaccctgcctcccagccgggaagaaatgaccaagaaccaggtgtccctgacctgtctggtggagggcttctacccttccgacatcgccgttgagtgggagtctaacggacagccggagaacaactacaagactacgcctccaatgctggactccgacggctccttcttcctgtactccgaactgaccgtggacaagtcccggtggcagcagggcaacgtgttctcatgctccgtaatgcacgaagccttgcacaatcactacactcaaaagtccctatccttatctcctggcaagtag

SEQ ID NO: 75 - DNA, 1395 bp, Artificial Sequence
  21M18 Heavy chain
atgaagcacctatggttctttctattattagtggccgctccccgttgggtgttatcgcaggttcagctagttcagtctggagcggaagttaagaaacctggagcatccgtgaaaataagttgcaaggcatccggttactcgttcaccgcatactatatccactgggttaaacaggcaccaggacagggacttgaatggatcggatatatctcctcttataatggagctacaaactataaccaaaaattcaaaggacgcgtgactttcacaactgacacctcaacctcgacagcatacatggaattacggtccctacggtctgacgacactgccgtttactattgcgctagagattatgattatgatgttggaatggactattggggccagggaacactggtgacagtgtcttctgcatccactaagggaccatccgtgttccctttggccccttgctctcgttcgacctctgaatcgactgccgctctgggatgcctcgtgaaagattacttccctgagcctgtgaccgtttcctggaactcgggcgccctaacctctggcgtgcacacattccctgccgtgctacagtcttctggcctatactctttatcttcggttgttaccgtaccttcttctaacttcggaacccaaacttacacctgtaacgtagaccacaagccttcgaacaccaaggtggacaagactgttgagcgaaagtgctgcgttgagtgccctccatgtcctgcacctcctgtggctggcccttctgtgttcctgttccctccaaaacctaaggacactctaatgatctctcggactcctgaggtgacttgcgtggttgtggacgtgtcccacgaggaccctgaggtgcagttcaattggtacgtggacggagtcgaggtgcacaatgcaaagaccaagcctcgggaggaacagttcaactccaccttccgggtggtttctgtgttgaccgttgtgcaccaagactggctgaacggcaaagaatacaagtgcaaggtgtccaacaagggcctgcctgcccctatcgaaaagaccatcagcaagaccaagggccagcctcgcgagcctcaggtgtacaccctgcctcccagccgggaagaaatgaccaagaaccaggtgtccctgacctgtctggtggagggcttctacccttccgacatcgccgttgagtgggagtctaacggacagccggagaacaactacaagactacgcctccaatgctggactccgacggctccttcttcctgtactccgaactgaccgtggacaagtcccggtggcagcagggcaacgtgttctcatgctccgtaatgcacgaagccttgcacaatcactacactcaaaagtccctatccttatctcctggcaagtag

SEQ ID NO: 76 - protein, 351 aa, Artificial Sequence
  21M18 Heavy chain variable region
CAGCTAGTTCAGTCTGGAGCGGAAGTTAAGAAACCTGGAGCATCCGTGAAAATAAGTTGCAAGGCATCCGGTTACTCGTTCACCGCATACTATATCCACTGGGTTAAACAGGCACCAGGACAGGGACTTGAATGGATCGGATATATCTCCTCTTATAATGGAGCTACAAACTATAACCAAAAATTCAAAGGACGCGTGACTTTCACAACTGACACCTCAACCTCGACAGCATACATGGAATTACGGTCCCTACGGTCTGACGACACTGCCGTTTACTATTGCGCTAGAGATTATGATTATGATGTTGGAATGGACTATTGGGGCCAGGGAACACTGGTGACAGTGTCTTCT

SEQ ID NO: 77 - DNA, 1392 bp, Artificial Sequence
  21R75 Heavy chain
  sig_peptide (1)..(57)
atgaagcacctgtggttctttctgctgctggtggccgctcccagatgggtgctgtctcaggtgcagctggtgcagtctggcgccgaagtgaagaaacctggcgcctccgtgaagatctcctgcaaggcctccggctactccttcaccgcctactacatccactgggtcaagcaggcccctggacagggcctggaatggatcggctatatcgccggctacaaggacgccaccaactacaaccagaaattcaagggcagagtgaccttcaccaccgacacctccacctctaccgcctacatggaactgcggtccctgcggagcgacgacaccgccgtgtactactgcgccagagactacgactacgacgtgggcatggactactggggccagggcacactcgtgaccgtgtcctctgcttccaccaagggcccctccgtgtttcctctggccccttgctccagatccacctccgagtctaccgccgctctgggctgcctcgtgaaggactacttccccgagcccgtgacagtgtcttggaactctggcgccctgacctccggcgtgcacacctttccagctgtgctgcagtcctccggcctgtactccctgtcctccgtcgtgactgtgccctcctccaacttcggcacccagacctacacctgtaacgtggaccacaagccctccaacaccaaggtggacaagaccgtggaacggaagtgctgcgtggaatgccccccttgtcctgcccctcctgtggctggccctagcgtgttcctgttccccccaaagcccaaggacaccctgatgatctcccggacccccgaagtgacctgcgtggtggtggatgtgtcccacgaggaccccgaggtgcagttcaattggtacgtggacggcgtggaagtgcacaacgccaagaccaagcccagagaggaacagttcaactccaccttccgggtggtgtccgtgctgaccgtggtgcatcaggactggctgaacggcaaagagtacaagtgcaaggtgtccaacaagggcctgcctgcccccatcgaaaagaccatctctaagaccaagggacagccccgcgagccccaggtgtacacactgcctccatcccgggaagagatgaccaagaaccaggtgtccctgacctgtctggtggaaggcttctacccctccgatatcgccgtggaatgggagtccaacggccagcccgagaacaactacaagaccaccccccccatgctggactccgacggctcattcttcctgtacagcgagctgacagtggacaagtcccggtggcagcagggcaacgtgttctcctgctccgtgatgcacgaggccctgcacaaccactacacccagaagtccctgtccctgagccccggcaag

SEQ ID NO: 78 - DNA, 1392 bp, Artificial Sequence
  21R83 Heavy chain
  sig_peptide (1)..(57)
atgaagcacctgtggttctttctgctgctggtggccgctcccagatgggtgctgtctcaggtgcagctggtgcagtctggcgccgaagtgaagaaacctggcgcctccgtgaagatctcctgcaaggcctccggctactccttcaccgcctactacatccactgggtcaagcaggcccctggacagggcctggaatggatcggctacatctccaactacaaccgggccaccaattacaaccagaaattcaagggccgcgtgaccttcaccaccgacacctctacctctaccgcctacatggaactgcggtccctgcggagcgacgacaccgccgtgtactactgcgccagagactacgactacgacgtgggcatggactactggggccagggcacactcgtgaccgtgtctagcgcttccaccaagggcccctccgtgtttcctctggccccttgctccagatccacctccgagtctaccgccgctctgggctgcctcgtgaaggactacttccccgagcccgtgacagtgtcctggaactctggcgctctgacctccggcgtgcacacctttccagctgtgctgcagtcctccggcctgtactccctgtcctccgtcgtgactgtgccctcctccaacttcggcacccagacctacacctgtaacgtggaccacaagccctccaacaccaaggtggacaagaccgtggaacggaagtgctgcgtggaatgccccccttgtcctgcccctcctgtggctggccctagcgtgttcctgttccccccaaagcccaaggacaccctgatgatctcccggacccccgaagtgacctgcgtggtggtggatgtgtcccacgaggaccccgaggtgcagttcaattggtacgtggacggcgtggaagtgcacaacgccaagaccaagcccagagaggaacagttcaactccaccttccgggtggtgtccgtgctgaccgtggtgcatcaggactggctgaacggcaaagagtacaagtgcaaggtgtccaacaagggcctgcctgcccccatcgaaaagaccatctctaagaccaagggacagccccgcgagccccaggtgtacacactgcctccatcccgggaagagatgaccaagaaccaggtgtccctgacctgtctggtggaaggcttctacccctccgatatcgccgtggaatgggagtccaacggccagcccgagaacaactacaagaccaccccccccatgctggactccgacggctcattcttcctgtacagcgagctgacagtggacaagtcccggtggcagcagggcaacgtgttctcctgctccgtgatgcacgaggccctgcacaaccactacacccagaagtccctgtccctgagccccggcaag

SEQ ID NO: 79 - protein, 5 aa, Artificial Sequence
  Alternative 21R75, 21R79, 21R83, and 21M18 Heavy chain CDR1
AYYIH

SEQ ID NO: 80 - protein, 17 aa, Artificial Sequence
  Anti-DLL4 heavy chain CDR2 consensus sequence
  MISC_FEATURE (3)..(3): X can be serine or alanine
  MISC_FEATURE (4)..(4): X can be serine, asparagine, or glycine
  MISC_FEATURE (6)..(6): X can be asparagine or lysine
  MISC_FEATURE (7)..(7): X can be glycine, arginine, or aspartic acid
YIXXYXXATNYNQKFKG